European Patent Application EP 4 538 384 A1, published April 16, 2025. Title: DETECTION METHOD AND DETECTION REAGENT FOR UNDIFFERENTIATED PLURIPOTENT STEM CELLS. Applicant: Kyoto University. Application WO PCT/JP2023/021545, filed June 9, 2023. The sequence listing filed with the application follows.

SEQUENCE LISTING (42 sequences)

SEQ ID NO: 1 - RNA, 395 nt, Homo sapiens
  source 1..395: mol_type = other RNA
taggaattctgctttaacttgttcctgcttgtggtgcatactacagaatgaaattaacagctctaaatactctgaagtccaaagaagttgtatgttgggtgggctcccttcaactttaacatggaagtgctttctgtgactttaaaagatctggacttacctcaattgcttttgctgcttgttcttttgtttcaaattccacaaacgcaaatccctttggatctccagtagacttataatgtggtatacttatataaacaacattgccacatttcccaaatactctttcaatccagctgtgattaacatttttgggaagtaactcctattataaattaaaagcaatattagagtttttcacaatcagaatgtcaataaatttttaacttaattat

SEQ ID NO: 2 - RNA, 351 nt, Homo sapiens
  source 1..351: mol_type = other RNA
ttttacccttctggaggagaacacgaatctttgggaactagttcaggaagggattctgcatcttcagagctgcttctcttcctcttccctgttctgacttcaggatctggacttacctcaattgcttttgctgcttgttcttttgtttcaaattccacaaacgcaaatccctttggatctccagtagacttataatgtggtatacttatataaacaacattgccacatttcccaaatactctttcaatccagctgtgattaacatttttgggaagtaactcctattataaattaaaagcaatattagagtttttcacaatcagaatgtcaataaatttttaacttaattat

SEQ ID NO: 3 - RNA, 298 nt, Homo sapiens
  source 1..298: mol_type = other RNA
ttttacccttctggaggagaacacgaatctttgggaactagttcaggaaggatctggacttacctcaattgcttttgctgcttgttcttttgtttcaaattccacaaacgcaaatccctttggatctccagtagacttataatgtggtatacttatataaacaacattgccacatttcccaaatactctttcaatccagctgtgattaacatttttgggaagtaactcctattataaattaaaagcaatattagagtttttcacaatcagaatgtcaataaatttttaacttaattat

SEQ ID NO: 4 - DNA, 20 bp, synthetic construct
  misc_feature 1..20: note = primer
  source 1..20: mol_type = other DNA
cccttctggaggagaacacg

SEQ ID NO: 5 - DNA, 21 bp, synthetic construct
  misc_feature 1..21: note = primer
  source 1..21: mol_type = other DNA
ggagatccaaagggatttgcg

SEQ ID NO: 6 - DNA, 20 bp, synthetic construct
  misc_feature 1..20: note = primer
  source 1..20: mol_type = other DNA
ccttctggaggagaacacga

SEQ ID NO: 7 - DNA, 21 bp, synthetic construct
  misc_feature 1..21: note = primer
  source 1..21: mol_type = other DNA
agcagcaaaagcaattgaggt

SEQ ID NO: 8 - DNA, 20 bp, synthetic construct
  misc_feature 1..20: note = primer
  source 1..20: mol_type = other DNA
acccttctggaggagaacac

SEQ ID NO: 9 - DNA, 20 bp, synthetic construct
  misc_feature 1..20: note = primer
  source 1..20: mol_type = other DNA
agggatttgcgtttgtggaa

SEQ ID NO: 10 - DNA, 21 bp, synthetic construct
  misc_feature 1..21: note = primer
  source 1..21: mol_type = other DNA
ccttctggaggagaacacgaa

SEQ ID NO: 11 - DNA, 20 bp, synthetic construct
  misc_feature 1..20: note = primer
  source 1..20: mol_type = other DNA
aagggatttgcgtttgtgga

SEQ ID NO: 12 - DNA, 21 bp, synthetic construct
  misc_feature 1..21: note = primer
  source 1..21: mol_type = other DNA
cccttctggaggagaacacga

SEQ ID NO: 13 - DNA, 21 bp, synthetic construct
  misc_feature 1..21: note = primer
  source 1..21: mol_type = other DNA
aagggatttgcgtttgtggaa

SEQ ID NO: 14 - DNA, 21 bp, synthetic construct
  misc_feature 1..21: note = primer
  source 1..21: mol_type = other DNA
ccttctggaggagaacacgaa

SEQ ID NO: 15 - DNA, 21 bp, synthetic construct
  misc_feature 1..21: note = primer
  source 1..21: mol_type = other DNA
gaggaagagaagcagctctga

SEQ ID NO: 16 - DNA, 21 bp, synthetic construct
  misc_feature 1..21: note = primer
  source 1..21: mol_type = other DNA
acccttctggaggagaacacg

SEQ ID NO: 17 - DNA, 22 bp, synthetic construct
  misc_feature 1..22: note = primer
  source 1..22: mol_type = other DNA
agcagctctgaagatgcagaat

SEQ ID NO: 18 - DNA, 22 bp, synthetic construct
  misc_feature 1..22: note = primer
  source 1..22: mol_type = other DNA
ccctgttctgacttcaggatct

SEQ ID NO: 19 - DNA, 23 bp, synthetic construct
  misc_feature 1..23: note = primer
  source 1..23: mol_type = other DNA
gggatttgcgtttgtggaatttg

SEQ ID NO: 20 - DNA, 21 bp, synthetic construct
  misc_feature 1..21: note = primer
  source 1..21: mol_type = other DNA
aggagaacacgaatctttggg

SEQ ID NO: 21 - DNA, 22 bp, synthetic construct
  misc_feature 1..22: note = primer
  source 1..22: mol_type = other DNA
gaggaagagaagcagctctgaa

SEQ ID NO: 22 - DNA, 22 bp, synthetic construct
  misc_feature 1..22: note = primer
  source 1..22: mol_type = other DNA
ttctggaggagaacacgaatct

SEQ ID NO: 23 - DNA, 21 bp, synthetic construct
  misc_feature 1..21: note = primer
  source 1..21: mol_type = other DNA
aggaagagaagcagctctgaa

SEQ ID NO: 24 - DNA, 23 bp, synthetic construct
  misc_feature 1..23: note = primer
  source 1..23: mol_type = other DNA
cttctggaggagaacacgaatct

SEQ ID NO: 25 - DNA, 22 bp, synthetic construct
  misc_feature 1..22: note = primer
  source 1..22: mol_type = other DNA
agaggaagagaagcagctctga

SEQ ID NO: 26 - DNA, 23 bp, synthetic construct
  misc_feature 1..23: note = primer
  source 1..23: mol_type = other DNA
gaggagaacacgaatctttggga

SEQ ID NO: 27 - DNA, 22 bp, synthetic construct
  misc_feature 1..22: note = primer
  source 1..22: mol_type = other DNA
tgaagtcagaacagggaagagg

SEQ ID NO: 28 - DNA, 23 bp, synthetic construct
  misc_feature 1..23: note = primer
  source 1..23: mol_type = other DNA
actagttcaggaagggattctgc

SEQ ID NO: 29 - DNA, 22 bp, synthetic construct
  misc_feature 1..22: note = primer
  source 1..22: mol_type = other DNA
gatcctgaagtcagaacaggga

SEQ ID NO: 30 - DNA, 22 bp, synthetic construct
  misc_feature 1..22: note = primer
  source 1..22: mol_type = other DNA
ggagaacacgaatctttgggaa

SEQ ID NO: 31 - DNA, 22 bp, synthetic construct
  misc_feature 1..22: note = primer
  source 1..22: mol_type = other DNA
cctgaagtcagaacagggaaga

SEQ ID NO: 32 - DNA, 22 bp, synthetic construct
  misc_feature 1..22: note = primer
  source 1..22: mol_type = other DNA
tcaggaagggattctgcatctt

SEQ ID NO: 33 - DNA, 23 bp, synthetic construct
  misc_feature 1..23: note = primer
  source 1..23: mol_type = other DNA
gtccagatcctgaagtcagaaca

SEQ ID NO: 34 - DNA, 18 bp, synthetic construct
  misc_feature 1..18: note = primer
  source 1..18: mol_type = other DNA
ctgcttctcttcctcttc

SEQ ID NO: 35 - DNA, 18 bp, synthetic construct
  misc_feature 1..18: note = primer
  source 1..18: mol_type = other DNA
gcgtttgtggaatttgaa

SEQ ID NO: 36 - DNA, 27 bp, synthetic construct
  misc_feature 1..27: note = probe
  source 1..27: mol_type = other DNA
acttcaggatctggacttacctcaatt

SEQ ID NO: 37 - DNA, 20 bp, synthetic construct
  misc_feature 1..20: note = primer
  source 1..20: mol_type = other DNA
gaaacccacactgcagcaga

SEQ ID NO: 38 - DNA, 18 bp, synthetic construct
  misc_feature 1..18: note = primer
  source 1..18: mol_type = other DNA
tcgcttgcccttctggcg

SEQ ID NO: 39 - DNA, 22 bp, synthetic construct
  misc_feature 1..22: note = primer
  source 1..22: mol_type = other DNA
atggagcttgtaagaaggctca

SEQ ID NO: 40 - DNA, 21 bp, synthetic construct
  misc_feature 1..21: note = primer
  source 1..21: mol_type = other DNA
gagttgcaggatcatggcttt

SEQ ID NO: 41 - DNA, 22 bp, synthetic construct
  misc_feature 1..22: note = primer
  source 1..22: mol_type = other DNA
gagccaagagtgaagaacagtc

SEQ ID NO: 42 - DNA, 23 bp, synthetic construct
  misc_feature 1..23: note = primer
  source 1..23: mol_type = other DNA
gctccccaccatattctgaatct